European Patent Application EP 4 582 547 A1, published July 9, 2025. Title: METHOD FOR FERMENTATIVELY PRODUCING L-GLUTAMIC ACID DERIVED FROM NITROGEN MOLECULES. Applicant: Kikkoman Corporation. Application EP 23860423.5, filed August 30, 2023. The sequence listing filed with the application follows.

SEQUENCE LISTING (45 sequences)

SEQ ID NO: 1 - DNA, 1305 bp, Klebsiella oxytoca
  source 1..1305: mol_type = other DNA
  CDS 13..1296: protein_id = 28; translation = MSDAKAKITLGGDTAIELDVLKGTLGQDVIDIRSLGSKGVFTFDPGFTSTASCESKITFIDGDEGILLHRGFPIDQLATDSNYLEVCYILLNGEKPTQAQYDEFKTIVTRHTMIHEQITRLFHAFRRDSHPMAVMCGITGALAAFYHDSLDVNNPRHRDIAAFRLLSKMPTMAAMCYKYSIGQPFVYPRNDLSYAGNFLNMMFSTPCEKYEVNPILERAMDRILILHADHEQNASTSTVRTAGSSGANPFACIAAGIASLWGPAHGGANEAALKMLEEISSVEHIPEFVRRAKDKNDSFRLMGFGHRVYKNYDPRATVMRETCHEVLKELGTKDDLLEVAMELEHIALNDPYFIEKKLYPNVDFYSGIILKAMGIPSSMFTVIFAMARTVGWIAHWNEMHSDGMKIARPRQLYTGYEKRDFKNDIAR
aggagaccataaatgtctgatgctaaagcaaaaatcaccctgggtggtgatactgctatcgaactggatgtgctaaagggcacgctcggtcaggatgttattgatattcgtagtcttggttcaaaaggcgtatttacttttgaccctggtttcacctcaaccgcatcctgcgaatctaaaatcacctttatcgacggtgatgaaggtatcctgctgcaccgcggttttccgatcgatcagttagcaaccgactccaactatctggaagtatgctacatcctgctgaacggtgagaagccgactcaggcccagtacgacgaattcaaaacaatcgttactcgccacactatgattcacgaacagattacccgtctgttccacgcgttccgccgcgattcacatccgatggccgttatgtgcggtatcaccggcgcgctggccgcgttctatcacgattcgctggatgtgaataacccacgccatcgcgatatcgccgcattccgcctgctctccaagatgccgacgatggcggcaatgtgttacaaatattctatcggtcagcctttcgtttatccgcgcaacgacctctcctacgcgggtaacttcctgaatatgatgttctccacgccgtgtgaaaaatatgaagtgaacccgattctggaacgcgcgatggaccgtatcctgatcctgcacgccgaccacgaacaaaacgcttcgacctccaccgtgcgtaccgccggctcttccggcgcgaacccgtttgcctgcatcgcagcgggcattgcctccctgtggggaccggcgcacggcggcgccaacgaagcggcgctgaagatgctcgaagagatcagctccgttgaacacattccggaattcgttcgtcgcgcgaaagacaaaaacgactctttccgcctgatgggctttggccaccgggtgtacaaaaactacgacccgcgcgccaccgttatgcgtgaaacctgccatgaagtgctgaaagagctgggcaccaaagacgatctgctggaagtggctatggagcttgagcacatcgcgcttaacgacccgtacttcattgagaagaaactttaccctaacgtcgatttctactccggtatcatcctcaaagcgatgggcatcccatcctccatgtttaccgttatcttcgcgatggcgcgtaccgtgggctggattgcgcactggaacgaaatgcacagcgacggcatgaaaatagcccgtccgcgtcagctgtataccggctacgaaaagcgcgatttcaaaaacgatatcgcccgctaagtcggctat

SEQ ID NO: 2 - DNA, 1442 bp, Klebsiella oxytoca
  source 1..1442: mol_type = other DNA
  CDS 52..1392: protein_id = 29; translation = MTNMSQAPSAEKKGVSDILGFKIFGMPLPLYAFALITLLLSHFYNALPTDIVGGFAIMFIIGAVFGEIGKRLPIFNKYIGGAPVMIFLVAAYFVYAGIFTQKEIDAITNVMDKSNFLNLFIAVLITGAILSVNRKLLLKSLLGYIPTILMGILGASIFGILIGLCFGISIDRIMMLYVLPIMGGGNGAGAVPLSEIYHSVTGRSREEYYSTAIAILTIANIFAIVFAALLDIIGKKHTWLSGEGELVRKASFKVEDDEKAGQITHRETAVGLVLATTCFLLAYVIAKKILPSIGGVSIHYFAWMVLIVAALNASGLCSPEIKAGAKRLSDFFSKQLLWVLMVGVGVCYTDLQEIIDAITFANVIIAAVIVVGAVIGAAIGGWMIGFFPIESAITAGLCMANRGGSGDLEVLSACNRMNLISYAQISSRLGGGIVLVIASIVFGMMM
gcagtttgaaggatgatgtgtatattcctttttttaacagggtgacgtcatatgactaatatgagccaggctccatctgcagagaaaaaaggcgttagcgatattctggggtttaaaatcttcggcatgccgctaccgctttacgcctttgcgttaatcactttactactttcacacttttataatgccctgccgaccgacattgtcggcggcttcgccatcatgtttattattggcgccgtttttggagaaattggcaaacgcctgccgatcttcaataaatatatcggcggcgcgccggtgatgatcttcctcgtggccgcctatttcgtttatgcaggcattttcacccagaaagaaattgatgcgatcactaatgtgatggataaaagtaacttcctgaacttattcatcgcagtattgattactggtgcaatcctctcggttaaccgtaagctgctgctgaaatctctgctgggttatattccgaccattttaatggggatcctcggcgcatccatcttcgggattctcatcggcttgtgcttcggtatctccatcgaccgcattatgatgctgtacgtcctgccgattatgggtggcggcaacggcgcgggcgcggtgccgctatctgaaatttatcactccgtcaccggccgttcgcgtgaagagtactactccaccgcgattgctatcctgaccatcgccaacatctttgccatcgtgtttgccgcgctgctcgatattatcggtaaaaagcacacctggctgagcggcgaaggcgagctggtgcgcaaggcctctttcaaagtagaagatgatgaaaaagcgggccagattacccatcgcgaaacggccgtcggcctggtgctcgccacaacctgcttcctgctggcctacgttatcgccaagaaaattctgccaagcattggcggcgtatctatccactatttcgcctggatggtgctgatcgtcgcggcgctgaacgcttccggcctctgctcgcctgagattaaagctggcgctaaacgcctatctgacttcttctctaagcaactgctgtgggtactgatggtcggcgtcggcgtgtgctacaccgacctgcaggaaattatcgacgcgattacctttgcgaacgtcatcatcgcggcggtgatcgtcgtgggcgcggtcatcggcgcggccatcggcggctggatgattggcttcttcccgattgaatccgcgatcaccgccggtctgtgcatggctaaccgcggcggctcgggcgacctggaagtactctctgcctgtaaccgtatgaatcttatctcttatgcgcaaatctcctcccgtctgggcggcggtattgtgctggtcattgccagcatcgtgttcggcatgatgatgtaaccaacacgcacgatggcgatgtttgagcgtcaaccacagcggtgctattt

SEQ ID NO: 3 - DNA, 1314 bp, Corynebacterium glutamicum
  source 1..1314: mol_type = other DNA
  CDS 1..1314: protein_id = 30; translation = MFERDIVATDNNKAVLHYPGGEFEMDIIEASEGNNGVVLGKMLSETGLITFDPGYVSTGSTESKITYIDGDAGILRYRGYDIADLAENATFNEVSYLLINGELPTPDELHKFNDEIRHHTLLDEDFKSQFNVFPRDAHPMATLASSVNILSTYYQDQLNPLDEAQLDKATVRLMAKVPMLAAYAHRARKGAPYMYPDNSLNARENFLRMMFGYPTEPYEIDPIMVKALDKLLILHADHEQNCSTSTVRMIGSAQANMFVSIAGGINALSGPLHGGANQAVLEMLEDIKNNHGGDATAFMNKVKNKEDGVRLMGFGHRVYKNYDPRAAIVKETAHEILEHLGGDDLLDLAIKLEEIALADDCFISRKLYPNVDFYTGLIYRAMGFPTDFFTVLFAIGRLPGWIAHYREQLGAAGNKINRPRQVYTGKESRKLVPREER
atgtttgaaagggatatcgtggctactgataacaacaaggctgtcctgcactaccccggtggcgagttcgaaatggacatcatcgaggcttctgagggtaacaacggtgttgtcctgggcaagatgctgtctgagactggactgatcacttttgacccaggttatgtgagcactggctccaccgagtcgaagatcacctacatcgatggcgatgcgggaatcctgcgttaccgcggctatgacatcgctgatctggctgagaatgccaccttcaacgaggtttcttacctacttatcaacggtgagctaccaaccccagatgagcttcacaagtttaacgacgagattcgccaccacacccttctggacgaggacttcaagtcccagttcaacgtgttcccacgcgacgctcacccaatggcaaccttggcttcctcggttaacattttgtctacctactaccaggatcagctgaacccactcgatgaggcacagcttgataaggcaaccgttcgcctcatggcaaaggttccaatgctggctgcgtacgcacaccgcgcacgcaagggtgctccttacatgtacccagacaactccctcaacgcgcgtgagaacttcctgcgcatgatgttcggttacccaaccgagccatacgagatcgacccaatcatggtcaaggctctggacaagctgctcatcctgcacgctgaccacgagcagaactgctccacctccaccgttcgtatgatcggttccgcacaggccaacatgtttgtctccatcgctggtggcatcaacgctctgtccggcccactgcacggtggcgcaaaccaggctgttctggagatgctcgaagacatcaagaacaaccacggtggcgacgcaaccgcgttcatgaacaaggtcaagaacaaggaagacggcgtccgcctcatgggcttcggacaccgcgtttacaagaactacgatccacgtgcagcaatcgtcaaggagaccgcacacgagatcctcgagcacctcggtggcgacgatcttctggatctggcaatcaagctggaagaaattgcactggctgatgattgcttcatctcccgcaagctctacccgaacgtagacttctacaccggcctgatctaccgcgcaatgggcttcccaactgacttcttcaccgtattgttcgcaatcggtcgtctgccaggatggatcgctcactaccgcgagcagctcggtgcagcaggcaacaagatcaaccgcccacgccaggtctacaccggcaaggaatcccgcaagttggttcctcgcgaggagcgctaa

SEQ ID NO: 4 - DNA, 1152 bp, Corynebacterium glutamicum
  source 1..1152: mol_type = other DNA
  CDS 1..1152: protein_id = 31; translation = MSSATTTDVRKGLYGVIADYTAVSKVMPETNSLTYRGYAVEDLVENCSFEEVFYLLWHGELPTAQQLAEFNERGRSYRSLDAGLISLIHSLPKEAHPMDVMRTAVSYMGTKDSEYFTTDSEHIRKVGHTLLAQLPMVLAMDIRRRKGLDIIAPDSSKSVAENLLSMVFGTGPESPASNPADVRDFEKSLILYAEHSFNASTFTARVITSTKSDVYSAITGAIGALKGPLHGGANEFVMHTMLAIDDPNKAADWINNALDNKNVVMGFGHRVYKRGDSRVPSMEKSFRELAARHDGEKWVAMYENMRDAMDARTGIKPNLDFPAGPAYHLLGFPVDFFTPLFVIARVAGWTAHIVEQYENNSLIRPLSEYNGEEQREVAPIEKR
atgtccagcgccacaaccactgatgttcgcaaaggactctacggagtcatcgcggattacacggccgtttccaaagtcatgccagagaccaattcactgacctaccgtggctacgcggtggaagatttggtggaaaactgcagcttcgaggaggtgttttacctcctgtggcacggcgagctgcccactgcgcaacaacttgcggagttcaatgagcgtggccgttcctaccgctccctggatgccggtttgatctccctgatccactctttgcccaaagaagcccacccgatggatgttatgcgcaccgcggtgtcctacatgggcaccaaggattccgagtatttcaccaccgattctgagcacatccgcaaagtcggccacaccttgttggcgcagcttccgatggtgctagccatggatattcgtcgccgcaagggcctcgatatcatcgcccctgactccagcaagtcagtcgccgaaaacctgctgtctatggtgtttggcaccggcccggagtcgcctgcatctaacccagctgacgtccgcgattttgagaaatcactgatcctctacgccgagcactccttcaacgcctccaccttcaccgcccgcgtgatcacctccaccaaatcggatgtgtactccgcaatcaccggcgcgatcggtgctctcaagggcccattgcacggtggcgccaacgagtttgtcatgcacaccatgttggcgatcgacgatcccaacaaggccgccgactggatcaacaacgctttggacaacaagaatgtggtcatgggctttggccaccgcgtgtacaagcgcggcgattcccgcgtgccatcgatggagaagtccttccgggaattagctgcccgccacgacggcgaaaagtgggttgccatgtatgaaaacatgcgcgacgccatggacgcccgcaccggcatcaagccgaatctcgatttccccgctggccctgcctaccacctgctcggcttcccggtcgatttcttcaccccgctgttcgtcatcgcgcgcgtcgccggctggaccgcacacatcgtggagcagtacgaaaacaactcgctcatccgcccactgtccgagtacaacggcgaggagcagcgcgaggtcgcgcccattgaaaagcgttaa

SEQ ID NO: 5 - DNA, 1170 bp, Escherichia coli
  source 1..1170: mol_type = other DNA
  CDS 1..1170: protein_id = 32; translation = MSDTTILQNSTHVIKPKKSVALSGVPAGNTALCTVGKSGNDLHYRGYDILDLAKHCEFEEVAHLLIHGKLPTRDELAAYKTKLKALRGLPANVRTVLEALPAASHPMDVMRTGVSALGCTLPEKEGHTVSGARDIADKLLASLSSILLYWYHYSHNGERIQPETDDDSIGGHFLHLLHGEKPSQSWEKAMHISLVLYAEHEFNASTFTSRVIAGTGSDMYSAIIGAIGALRGPKHGGANEVSLEIQQRYETPDEAEADIRKRVENKEVVIGFGHPVYTIADPRHQVIKRVAKQLSQEGGSLKMYNIADRLETVMWESKKMFPNLDWFSAVSYNMMGVPTEMFTPLFVIARVTGWAAHIIEQRQDNKIIRPSANYVGPEDRPFVALDKRQ
atgagcgacacaacgatcctgcaaaacagtacccatgtcattaaaccgaaaaaatctgtggcactttctggcgttccggcgggcaatacggcgctctgcaccgtgggtaaaagtggcaatgacctgcattaccgcggctacgatattcttgatctggcgaaacattgcgaatttgaagaagtggcgcatctgctgatccacggcaaactgccgacccgtgacgaactcgccgcttacaaaacgaaactgaaagccctgcgcggtttaccggctaacgtgcgtaccgtgctggaagccttaccggcggcgtcgcacccgatggatgttatgcgcaccggtgtttccgcgctcggctgcacgctgccagaaaaagaggggcataccgtctctggcgcgcgggatattgccgacaaactgctggcgtcgcttagctcgattctcctttattggtatcactacagccacaacggcgaacgcatccaaccggaaaccgatgacgactccatcggcggtcacttcctgcatctgctgcacggcgaaaagccatcgcaaagctgggaaaaggcgatgcatatctcgctggtgctgtacgccgaacacgagtttaacgcctccacctttaccagtcgggtgattgcgggcaccggctctgatatgtattccgcgattattggcgcgattggcgcactgcgcgggccaaaacacggcggggcgaatgaagtgtcgctggagatccagcaacgctacgaaacgccggacgaagccgaagcagatatccgcaagcgcgtggaaaacaaagaagtggtcattggttttggtcatccggtttacaccatcgctgacccgcgccaccaggtgattaaacgtgtggcgaagcagctctcgcaggaaggcggctcgctgaagatgtacaacatcgccgatcgcctggaaacggtgatgtgggagagcaaaaagatgttccccaatctcgactggttctctgctgtttcctacaacatgatgggcgttcccaccgagatgttcacaccactgtttgttatcgcccgcgtcaccggctgggcggcgcacattatcgaacaacgtcaggacaacaaaattatccgtccttccgccaattatgttggaccggaagaccgcccgtttgtcgcgctggataagcgccagtaa

SEQ ID NO: 6 - DNA, 20 bp, synthetic construct
  source 1..20: mol_type = other DNA
aaggatctaggtgaagatcc

SEQ ID NO: 7 - DNA, 20 bp, synthetic construct
  source 1..20: mol_type = other DNA
ggttattgtctcatgagcgg

SEQ ID NO: 8 - DNA, 38 bp, synthetic construct
  source 1..38: mol_type = other DNA
ccgctcatgagacaataaccaattctcatgtttgacag

SEQ ID NO: 9 - DNA, 40 bp, synthetic construct
  source 1..40: mol_type = other DNA
ggatcttcacctagatccttattcaggtcgaggtggcccg

SEQ ID NO: 10 - DNA, 24 bp, synthetic construct
  source 1..24: mol_type = other DNA
ggtttattcctccttatttaatcg

SEQ ID NO: 11 - DNA, 21 bp, synthetic construct
  source 1..21: mol_type = other DNA
aattcgaagcttacgtagaac

SEQ ID NO: 12 - DNA, 18 bp, synthetic construct
  source 1..18: mol_type = other DNA
ctcccgttctggataatg

SEQ ID NO: 13 - DNA, 38 bp, synthetic construct
  source 1..38: mol_type = other DNA
cgggtaccgagctcgaattcttagcgctcctcgcgagg

SEQ ID NO: 14 - DNA, 18 bp, synthetic construct
  source 1..18: mol_type = other DNA
gaattcgagctcggtacc

SEQ ID NO: 15 - DNA, 38 bp, synthetic construct
  source 1..38: mol_type = other DNA
cgggtaccgagctcgaattcttaacgcttttcaatggg

SEQ ID NO: 16 - DNA, 38 bp, synthetic construct
  source 1..38: mol_type = other DNA
cgggtaccgagctcgaattcttactggcgcttatccag

SEQ ID NO: 17 - DNA, 18 bp, synthetic construct
  source 1..18: mol_type = other DNA
catggactcgtctactag

SEQ ID NO: 18 - DNA, 38 bp, synthetic construct
  source 1..38: mol_type = other DNA
aacattatccagaacgggagtcctaatgcaggagtcgc

SEQ ID NO: 19 - DNA, 42 bp, synthetic construct
  source 1..42: mol_type = other DNA
cgattaaataaggaggaataaaccatgtttgaaagggatatc

SEQ ID NO: 20 - DNA, 38 bp, synthetic construct
  source 1..38: mol_type = other DNA
gggtgttggcgggtgtcgggcgctcactgcccgctttc

SEQ ID NO: 21 - DNA, 20 bp, synthetic construct
  source 1..20: mol_type = other DNA
cccgacacccgccaacaccc

SEQ ID NO: 22 - DNA, 42 bp, synthetic construct
  source 1..42: mol_type = other DNA
cgattaaataaggaggaataaaccatgtccagcgccacaacc

SEQ ID NO: 23 - DNA, 42 bp, synthetic construct
  source 1..42: mol_type = other DNA
cgattaaataaggaggaataaaccatgagcgacacaacgatc

SEQ ID NO: 24 - DNA, 44 bp, synthetic construct
  source 1..44: mol_type = other DNA
cgattaaataaggaggaataaaccatgactaatatgagccaggc

SEQ ID NO: 25 - DNA, 42 bp, synthetic construct
  source 1..42: mol_type = other DNA
cgattaaataaggaggaataaaccatgtctgatgctaaagca

SEQ ID NO: 26 - DNA, 39 bp, synthetic construct
  source 1..39: mol_type = other DNA
gttctacgtaagcttcgaattttagcgggcgatatcgtt

SEQ ID NO: 27 - DNA, 39 bp, synthetic construct
  source 1..39: mol_type = other DNA
cgctagtagacgagtccatgttacatcatcatgccgaac

SEQ ID NO: 28 - protein, 427 aa, Klebsiella oxytoca
MSDAKAKITLGGDTAIELDVLKGTLGQDVIDIRSLGSKGVFTFDPGFTSTASCESKITFIDGDEGILLHRGFPIDQLATDSNYLEVCYILLNGEKPTQAQYDEFKTIVTRHTMIHEQITRLFHAFRRDSHPMAVMCGITGALAAFYHDSLDVNNPRHRDIAAFRLLSKMPTMAAMCYKYSIGQPFVYPRNDLSYAGNFLNMMFSTPCEKYEVNPILERAMDRILILHADHEQNASTSTVRTAGSSGANPFACIAAGIASLWGPAHGGANEAALKMLEEISSVEHIPEFVRRAKDKNDSFRLMGFGHRVYKNYDPRATVMRETCHEVLKELGTKDDLLEVAMELEHIALNDPYFIEKKLYPNVDFYSGIILKAMGIPSSMFTVIFAMARTVGWIAHWNEMHSDGMKIARPRQLYTGYEKRDFKNDIAR

SEQ ID NO: 29 - protein, 446 aa, Klebsiella oxytoca
MTNMSQAPSAEKKGVSDILGFKIFGMPLPLYAFALITLLLSHFYNALPTDIVGGFAIMFIIGAVFGEIGKRLPIFNKYIGGAPVMIFLVAAYFVYAGIFTQKEIDAITNVMDKSNFLNLFIAVLITGAILSVNRKLLLKSLLGYIPTILMGILGASIFGILIGLCFGISIDRIMMLYVLPIMGGGNGAGAVPLSEIYHSVTGRSREEYYSTAIAILTIANIFAIVFAALLDIIGKKHTWLSGEGELVRKASFKVEDDEKAGQITHRETAVGLVLATTCFLLAYVIAKKILPSIGGVSIHYFAWMVLIVAALNASGLCSPEIKAGAKRLSDFFSKQLLWVLMVGVGVCYTDLQEIIDAITFANVIIAAVIVVGAVIGAAIGGWMIGFFPIESAITAGLCMANRGGSGDLEVLSACNRMNLISYAQISSRLGGGIVLVIASIVFGMMM

SEQ ID NO: 30 - protein, 437 aa, Corynebacterium glutamicum
MFERDIVATDNNKAVLHYPGGEFEMDIIEASEGNNGVVLGKMLSETGLITFDPGYVSTGSTESKITYIDGDAGILRYRGYDIADLAENATFNEVSYLLINGELPTPDELHKFNDEIRHHTLLDEDFKSQFNVFPRDAHPMATLASSVNILSTYYQDQLNPLDEAQLDKATVRLMAKVPMLAAYAHRARKGAPYMYPDNSLNARENFLRMMFGYPTEPYEIDPIMVKALDKLLILHADHEQNCSTSTVRMIGSAQANMFVSIAGGINALSGPLHGGANQAVLEMLEDIKNNHGGDATAFMNKVKNKEDGVRLMGFGHRVYKNYDPRAAIVKETAHEILEHLGGDDLLDLAIKLEEIALADDCFISRKLYPNVDFYTGLIYRAMGFPTDFFTVLFAIGRLPGWIAHYREQLGAAGNKINRPRQVYTGKESRKLVPREER

SEQ ID NO: 31 - protein, 383 aa, Corynebacterium glutamicum
MSSATTTDVRKGLYGVIADYTAVSKVMPETNSLTYRGYAVEDLVENCSFEEVFYLLWHGELPTAQQLAEFNERGRSYRSLDAGLISLIHSLPKEAHPMDVMRTAVSYMGTKDSEYFTTDSEHIRKVGHTLLAQLPMVLAMDIRRRKGLDIIAPDSSKSVAENLLSMVFGTGPESPASNPADVRDFEKSLILYAEHSFNASTFTARVITSTKSDVYSAITGAIGALKGPLHGGANEFVMHTMLAIDDPNKAADWINNALDNKNVVMGFGHRVYKRGDSRVPSMEKSFRELAARHDGEKWVAMYENMRDAMDARTGIKPNLDFPAGPAYHLLGFPVDFFTPLFVIARVAGWTAHIVEQYENNSLIRPLSEYNGEEQREVAPIEKR

SEQ ID NO: 32 - protein, 389 aa, Escherichia coli
MSDTTILQNSTHVIKPKKSVALSGVPAGNTALCTVGKSGNDLHYRGYDILDLAKHCEFEEVAHLLIHGKLPTRDELAAYKTKLKALRGLPANVRTVLEALPAASHPMDVMRTGVSALGCTLPEKEGHTVSGARDIADKLLASLSSILLYWYHYSHNGERIQPETDDDSIGGHFLHLLHGEKPSQSWEKAMHISLVLYAEHEFNASTFTSRVIAGTGSDMYSAIIGAIGALRGPKHGGANEVSLEIQQRYETPDEAEADIRKRVENKEVVIGFGHPVYTIADPRHQVIKRVAKQLSQEGGSLKMYNIADRLETVMWESKKMFPNLDWFSAVSYNMMGVPTEMFTPLFVIARVTGWAAHIIEQRQDNKIIRPSANYVGPEDRPFVALDKRQ

SEQ ID NO: 33 - DNA, 1239 bp, Klebsiella oxytoca
  source 1..1239: mol_type = genomic DNA
  CDS 1..1239: protein_id = 37; translation = MAEFSPERRFTRIDRLPPYVFNITAELKMAARRRGEDIIDFSMGNPDGATPPHIVEKLCTVAQRPDTHGYSTSRGIPRLRRAISRWYQERYNVEIDPESEAIVTIGSKEGLAHLMLATLDHGDTVLVPNPSYPIHIYGAVIAGAQVRSVPLVEGVDFFNELERAIRESYPKPKMMILGFPSNPTAQCVELEFFEKVVALAKRYDVLVVHDLAYADIVYDGWKAPSIMQVPGARDVAVEFFTLSKSYNMAGWRIGFMVGNKTLVNALARIKSYHDYGTFTPLQVAAIAALEGDQQCVRDIAEQYKRRRDVLVKGLHEAGWMVECPKASMYVWAKIPEQYAAMGSLEFAKKLLQDAKVCVSPGIGFGDYGDTHVRFALIENRDRIRQAVRGIKSMFRADGLLPASTKLTSESNE
atggctgaattcagtcctgaacgccgttttacgcgtatcgatcgtctccccccgtacgtttttaatatcactgctgagctgaaaatggctgcgcgacgccgcggcgaagatattattgatttcagcatgggtaaccccgatggcgcgaccccgccgcatatcgttgagaagctatgcaccgttgcccagcgtcccgatacgcacggctattccacctctcgcggtattccgcgtctgcgccgggcgatttctcgttggtatcaagagcgctataacgttgagatcgatccggaatcagaagcgatagtaaccattggttcaaaagagggactggcgcatctgatgctggcgacgcttgaccatggcgataccgtactggtgccgaatcccagctatcctattcacatttatggggcggtaatcgccggagcccaggtgcgttcagtacctctcgttgaaggcgtggattttttcaatgagctcgagcgcgccattcgcgagagttacccgaagccgaaaatgatgatcctcggtttcccttccaacccgaccgcgcagtgcgtcgaactggagttctttgagaaagtcgtggcgttggcgaagcgttatgacgtactggttgtgcacgatttggcctacgccgatattgtttatgatggctggaaagcgccctctattatgcaggttcccggcgcgcgcgatgttgccgtcgaattctttacgctatcgaaaagctacaatatggcgggctggcgtatcggctttatggttggcaacaaaacgttggttaatgcgctggcgcgtattaaaagctaccacgactacggcaccttcacccctctacaggttgcggctattgcggcgcttgaaggcgatcagcagtgcgttcgtgacattgccgagcagtataagcgccgtcgcgatgtgctggtgaaaggactgcatgaggccggatggatggtggaatgtccgaaggcgtcaatgtatgtatgggcgaagatccctgaacagtatgcggcgatgggctcactggagttcgctaaaaagctgctgcaggatgctaaagtctgcgtttcgccgggcattggcttcggggactacggcgatacgcacgtacgcttcgctttaattgaaaaccgcgatcgtatccgccaggcggtgcgcggcattaaatccatgtttcgtgcagacgggctgctgcccgcctcgacgaagttaaccagcgaaagcaacgaataa

SEQ ID NO: 34 - DNA, 456 bp, Klebsiella oxytoca
  source 1..456: mol_type = genomic DNA
  CDS 1..456: protein_id = 38; translation = MFSAQSRLRHAVADTFAMVVYCTVVNMMIEIFLSGMTFQQSLSSRLVAIPVNIIIAVPYGFYRDFAMRQARRISASGWMKNIADVVAYVTFQSPVYVAILLVVGADWHQIAAAVSSNIVVSMMMGAAYGYFLDYCRRLFRVSPLPAGQSLS
atgttctctgcgcagtcccgcttgcgtcatgcggtagcagacacctttgcgatggtggtttactgcaccgttgtgaacatgatgatcgaaatttttctctccggaatgaccttccagcagtcgttatcttcgcgactggtggcgattccggtgaacattattattgccgtgccttacggcttttatcgcgatttcgcgatgcgccaggcgcgccgcatcagcgcgtccggctggatgaagaatattgccgatgtagtggcctatgtgacgttccagtcgccggtatacgtggcgattctgctggttgttggcgccgactggcatcagatcgccgcggcggtaagttccaatatcgttgtatcaatgatgatgggcgcagcgtacggttatttcctcgactactgccgtcgcctgttccgcgtcagccccctacctgcaggccaaagcctgagttga

SEQ ID NO: 35 - DNA, 1191 bp, Escherichia coli
  source 1..1191: mol_type = genomic DNA
  CDS 1..1191: protein_id = 39; translation = MFENITAAPADPILGLADLFRADERPGKINLGIGVYKDETGKTPVLTSVKKAEQYLLENETTKNYLGIDGIPEFGRCTQELLFGKGSALINDKRARTAQTPGGTGALRVAADFLAKNTSVKRVWVSNPSWPNHKSVFNSAGLEVREYAYYDAENHTLDFDALINSLNEAQAGDVVLFHGCCHNPTGIDPTLEQWQTLAQLSVEKGWLPLFDFAYQGFARGLEEDAEGLRAFAAMHKELIVASSYSKNFGLYNERVGACTLVAADSETVDRAFSQMKAAIRANYSNPPAHGASVVATILSNDALRAIWEQELTDMRQRIQRMRQLFVNTLQEKGANRDFSFIIKQNGMFSFSGLTKEQVLRLREEFGVYAVASGRVNVAGMTPDNMAPLCEAIVAVL
atgtttgagaacattaccgccgctcctgccgacccgattctgggcctggccgatctgtttcgtgccgatgaacgtcccggcaaaattaacctcgggattggtgtctataaagatgagacgggcaaaaccccggtactgaccagcgtgaaaaaggctgaacagtatctgctcgaaaatgaaaccaccaaaaattacctcggcattgacggcatccctgaatttggtcgctgcactcaggaactgctgtttggtaaaggtagcgccctgatcaatgacaaacgtgctcgcacggcacagactccggggggcactggcgcactacgcgtggctgccgatttcctggcaaaaaataccagcgttaagcgtgtgtgggtgagcaacccaagctggccgaaccataagagcgtctttaactctgcaggtctggaagttcgtgaatacgcttattatgatgcggaaaatcacactcttgacttcgatgcactgattaacagcctgaatgaagctcaggctggcgacgtagtgctgttccatggctgctgccataacccaaccggtatcgaccctacgctggaacaatggcaaacactggcacaactctccgttgagaaaggctggttaccgctgtttgacttcgcttaccagggttttgcccgtggtctggaagaagatgctgaaggactgcgcgctttcgcggctatgcataaagagctgattgttgccagttcctactctaaaaactttggcctgtacaacgagcgtgttggcgcttgtactctggttgctgccgacagtgaaaccgttgatcgcgcattcagccaaatgaaagcggcgattcgcgctaactactctaacccaccagcacacggcgcttctgttgttgccaccatcctgagcaacgatgcgttacgtgcgatttgggaacaagagctgactgatatgcgccagcgtattcagcgtatgcgtcagttgttcgtcaatacgctgcaggaaaaaggcgcaaaccgcgacttcagctttatcatcaaacagaacggcatgttctccttcagtggcctgacaaaagaacaagtgctgcgtctgcgcgaagagtttggcgtatatgcggttgcttctggtcgcgtaaatgtggccgggatgacaccagataacatggctccgctgtgcgaagcgattgtggcagtgctgtaa

SEQ ID NO: 36 - DNA, 1401 bp, Escherichia coli
  source 1..1401: mol_type = genomic DNA
  CDS 1..1401: protein_id = 40; translation = MDKKQVTDLRSELLDSRFGAKSISTIAESKRFPLHEMRDDVAFQIINDELYLDGNARQNLATFCQTWDDENVHKLMDLSINKNWIDKEEYPQSAAIDLRCVNMVADLWHAPAPKNGQAVGTNTIGSSEACMLGGMAMKWRWRKRMEAAGKPTDKPNLVCGPVQICWHKFARYWDVELREIPMRPGQLFMDPKRMIEACDENTIGVVPTFGVTYTGNYEFPQPLHDALDKFQADTGIDIDMHIDAASGGFLAPFVAPDIVWDFRLPRVKSISASGHKFGLAPLGCGWVIWRDEEALPQELVFNVDYLGGQIGTFAINFSRPAGQVIAQYYEFLRLGREGYTKVQNASYQVAAYLADEIAKLGPYEFICTGRPDEGIPAVCFKLKDGEDPGYTLYDLSERLRLRGWQVPAFTLGGEATDIVVMRIMCRRGFEMDFAELLLEDYKASLKYLSDHPKLQGIAQQNSFKHT
atggataagaagcaagtaacggatttaaggtcggaactactcgattcacgttttggtgcgaagtctatttccactatcgcagaatcaaaacgttttccgctgcacgaaatgcgcgacgatgtcgcattccagattatcaatgacgaattatatcttgatggcaacgctcgtcagaacctggccactttctgccagacctgggacgacgaaaatgtccacaaattgatggatttatccattaacaaaaactggatcgacaaagaagaatatccgcaatccgcagccatcgacctgcgttgcgtaaatatggttgccgatctgtggcatgcgcctgcgccgaaaaatggtcaggccgttggcaccaacaccattggttcttccgaggcctgtatgctcggcgggatggcgatgaaatggcgttggcgcaagcgtatggaagctgcaggcaaaccaacggataaaccaaacctggtgtgcggtccggtacaaatctgctggcataaattcgcccgctactgggatgtggagctgcgtgagatccctatgcgccccggtcagttgtttatggacccgaaacgcatgattgaagcctgtgacgaaaacaccatcggcgtggtgccgactttcggcgtgacctacactggtaactatgagttcccacaaccgctgcacgatgcgctggataaattccaggccgataccggtatcgacatcgacatgcacatcgacgctgccagcggtggcttcctggcaccgttcgtcgccccggatatcgtctgggacttccgcctgccgcgtgtgaaatcgatcagtgcttcaggccataaattcggtctggctccgctgggctgcggctgggttatctggcgtgacgaagaagcgctgccgcaggaactggtgttcaacgttgactacctgggtggtcaaattggtacttttgccatcaacttctcccgcccggcgggtcaggtaattgcacagtactatgaattcctgcgcctcggtcgtgaaggctataccaaagtacagaacgcctcttaccaggttgccgcttatctggcggatgaaatcgccaaactggggccgtatgagttcatctgtacgggtcgcccggacgaaggcatcccggcggtttgcttcaaactgaaagatggtgaagatccgggatacaccctgtatgacctctctgaacgtctgcgtctgcgcggctggcaggttccggccttcactctcggcggtgaagccaccgacatcgtggtgatgcgcattatgtgtcgtcgcggcttcgaaatggactttgctgaactgttgctggaagactacaaagcctccctgaaatatctcagcgatcacccgaaactgcagggtattgcccaacagaacagctttaaacatacctga

SEQ ID NO: 37 - protein, 412 aa, Klebsiella oxytoca
MAEFSPERRFTRIDRLPPYVFNITAELKMAARRRGEDIIDFSMGNPDGATPPHIVEKLCTVAQRPDTHGYSTSRGIPRLRRAISRWYQERYNVEIDPESEAIVTIGSKEGLAHLMLATLDHGDTVLVPNPSYPIHIYGAVIAGAQVRSVPLVEGVDFFNELERAIRESYPKPKMMILGFPSNPTAQCVELEFFEKVVALAKRYDVLVVHDLAYADIVYDGWKAPSIMQVPGARDVAVEFFTLSKSYNMAGWRIGFMVGNKTLVNALARIKSYHDYGTFTPLQVAAIAALEGDQQCVRDIAEQYKRRRDVLVKGLHEAGWMVECPKASMYVWAKIPEQYAAMGSLEFAKKLLQDAKVCVSPGIGFGDYGDTHVRFALIENRDRIRQAVRGIKSMFRADGLLPASTKLTSESNE

SEQ ID NO: 38 - protein, 151 aa, Klebsiella oxytoca
MFSAQSRLRHAVADTFAMVVYCTVVNMMIEIFLSGMTFQQSLSSRLVAIPVNIIIAVPYGFYRDFAMRQARRISASGWMKNIADVVAYVTFQSPVYVAILLVVGADWHQIAAAVSSNIVVSMMMGAAYGYFLDYCRRLFRVSPLPAGQSLS

SEQ ID NO: 39 - protein, 396 aa, Escherichia coli
MFENITAAPADPILGLADLFRADERPGKINLGIGVYKDETGKTPVLTSVKKAEQYLLENETTKNYLGIDGIPEFGRCTQELLFGKGSALINDKRARTAQTPGGTGALRVAADFLAKNTSVKRVWVSNPSWPNHKSVFNSAGLEVREYAYYDAENHTLDFDALINSLNEAQAGDVVLFHGCCHNPTGIDPTLEQWQTLAQLSVEKGWLPLFDFAYQGFARGLEEDAEGLRAFAAMHKELIVASSYSKNFGLYNERVGACTLVAADSETVDRAFSQMKAAIRANYSNPPAHGASVVATILSNDALRAIWEQELTDMRQRIQRMRQLFVNTLQEKGANRDFSFIIKQNGMFSFSGLTKEQVLRLREEFGVYAVASGRVNVAGMTPDNMAPLCEAIVAVL

SEQ ID NO: 40 - protein, 466 aa, Escherichia coli
MDKKQVTDLRSELLDSRFGAKSISTIAESKRFPLHEMRDDVAFQIINDELYLDGNARQNLATFCQTWDDENVHKLMDLSINKNWIDKEEYPQSAAIDLRCVNMVADLWHAPAPKNGQAVGTNTIGSSEACMLGGMAMKWRWRKRMEAAGKPTDKPNLVCGPVQICWHKFARYWDVELREIPMRPGQLFMDPKRMIEACDENTIGVVPTFGVTYTGNYEFPQPLHDALDKFQADTGIDIDMHIDAASGGFLAPFVAPDIVWDFRLPRVKSISASGHKFGLAPLGCGWVIWRDEEALPQELVFNVDYLGGQIGTFAINFSRPAGQVIAQYYEFLRLGREGYTKVQNASYQVAAYLADEIAKLGPYEFICTGRPDEGIPAVCFKLKDGEDPGYTLYDLSERLRLRGWQVPAFTLGGEATDIVVMRIMCRRGFEMDFAELLLEDYKASLKYLSDHPKLQGIAQQNSFKHT

SEQ ID NO: 41 - DNA, 43 bp, synthetic construct
  source 1..43: mol_type = other DNA
cgattaaataaggaggaataaaccatggctgaattcagtcctg

SEQ ID NO: 42 - DNA, 41 bp, synthetic construct
  source 1..41: mol_type = other DNA
gtgctcctcgaaaatgaagtcgttattcgttgctttcgctg

SEQ ID NO: 43 - DNA, 19 bp, synthetic construct
  source 1..19: mol_type = other DNA
cgacttcattttcgaggag

SEQ ID NO: 44 - DNA, 38 bp, synthetic construct
  source 1..38: mol_type = other DNA
cgctagtagacgagtccatgtcaactcaggctttggcc

SEQ ID NO: 45 - DNA, 38 bp, synthetic construct
  source 1..38: mol_type = other DNA
ctagtagacgagtccatgttattcgttgctttcgctgg